European Patent Application EP 4 339 617 A1, published March 20, 2024. Title: ANALISIS METHOD FOR NEUROGRANIN-RELATED PEPTIDE. Applicant: SHIMADZU CORPORATION. The sequence listing filed with the application follows.

SEQUENCE LISTING (2 sequences)

SEQ ID NO: 1 - protein, 29 aa, Homo sapiens
ERGRKGPGPGGPGGAGVARGGAGGGPSGD

SEQ ID NO: 2 - protein, 33 aa, Homo sapiens
RKKIKSGERGRKGPGPGGPGGAGVARGGAGGGP